European Patent Application EP 4 450 087 A2, published October 23, 2024. Title: T CELL RECEPTORS AND IMMUNE THERAPY USING THE SAME AGAINST PRAME POSITIVE CANCERS. Applicant: Immatics Biotechnologies GmbH. Application EP. The sequence listing filed with the application follows.

SEQUENCE LISTING (204 sequences)

SEQ ID NO: 1 - protein, 6 aa, Homo sapiens
SSNFYA

SEQ ID NO: 2 - skipped

SEQ ID NO: 3 - protein, 11 aa, Homo sapiens
CALYNNNDMRF

SEQ ID NO: 4 - protein, 132 aa, Homo sapiens
MEKNPLAAPLLILWFHLDCVSSILNVEQSPQSLHVQEGDSTNFTCSFPSSNFYALHWYRWETAKSPEALFVMTLNGDEKKKGRISATLNTKEGYSYLYIKGSQPEDSATYLCALYNNNDMRFGAGTRLTVKP

SEQ ID NO: 5 - protein, 141 aa, Homo sapiens
NIQNPDPAVYQLRDSKSSDKSVCLFTDFDSQTNVSQSKDSDVYITDKTVLDMRSMDFKSNSAVAWSNKSDFACANAFNNSIIPEDTFFPSPESSCDVKLVEKSFETDTNLNFQNLSVIGFRILLLKVAGFNLLMTLRLWSS

SEQ ID NO: 6 - protein, 273 aa, Homo sapiens
MEKNPLAAPLLILWFHLDCVSSILNVEQSPQSLHVQEGDSTNFTCSFPSSNFYALHWYRWETAKSPEALFVMTLNGDEKKKGRISATLNTKEGYSYLYIKGSQPEDSATYLCALYNNNDMRFGAGTRLTVKPNIQNPDPAVYQLRDSKSSDKSVCLFTDFDSQTNVSQSKDSDVYITDKTVLDMRSMDFKSNSAVAWSNKSDFACANAFNNSIIPEDTFFPSPESSCDVKLVEKSFETDTNLNFQNLSVIGFRILLLKVAGFNLLMTLRLWSS

SEQ ID NO: 7 - protein, 5 aa, Homo sapiens
SGHNS

SEQ ID NO: 8 - protein, 6 aa, Homo sapiens
FNNNVP

SEQ ID NO: 9 - protein, 13 aa, Homo sapiens
CASSPGSTDTQYF

SEQ ID NO: 10 - protein, 132 aa, Homo sapiens
MDSWTFCCVSLCILVAKHTDAGVIQSPRHEVTEMGQEVTLRCKPISGHNSLFWYRQTMMRGLELLIYFNNNVPIDDSGMPEDRFSAKMPNASFSTLKIQPSEPRDSAVYFCASSPGSTDTQYFGPGTRLTVL

SEQ ID NO: 11 - protein, 179 aa, Homo sapiens
EDLKNVFPPEVAVFEPSEAEISHTQKATLVCLATGFYPDHVELSWWVNGKEVHSGVSTDPQPLKEQPALNDSRYCLSSRLRVSATFWQNPRNHFRCQVQFYGLSENDEWTQDRAKPVTQIVSAEAWGRADCGFTSESYQQGVLSATILYEILLGKATLYAVLVSALVLMAMVKRKDSRG

SEQ ID NO: 12 - protein, 311 aa, Homo sapiens
MDSWTFCCVSLCILVAKHTDAGVIQSPRHEVTEMGQEVTLRCKPISGHNSLFWYRQTMMRGLELLIYFNNNVPIDDSGMPEDRFSAKMPNASFSTLKIQPSEPRDSAVYFCASSPGSTDTQYFGPGTRLTVLEDLKNVFPPEVAVFEPSEAEISHTQKATLVCLATGFYPDHVELSWWVNGKEVHSGVSTDPQPLKEQPALNDSRYCLSSRLRVSATFWQNPRNHFRCQVQFYGLSENDEWTQDRAKPVTQIVSAEAWGRADCGFTSESYQQGVLSATILYEILLGKATLYAVLVSALVLMAMVKRKDSRG

SEQ ID NO: 13 - protein, 6 aa, Homo sapiens
DRGSQS

SEQ ID NO: 14 - skipped

SEQ ID NO: 15 - protein, 15 aa, Homo sapiens
CAAVISNFGNEKLTF

SEQ ID NO: 16 - protein, 134 aa, Homo sapiens
MKSLRVLLVILWLQLSWVWSQQKEVEQNSGPLSVPEGAIASLNCTYSDRGSQSFFWYRQYSGKSPELIMFIYSNGDKEDGRFTAQLNKASQYVSLLIRDSQPSDSATYLCAAVISNFGNEKLTFGTGTRLTIIP

SEQ ID NO: 17 - protein, 141 aa, Homo sapiens; identical to SEQ ID NO: 5

SEQ ID NO: 18 - protein, 275 aa, Homo sapiens
MKSLRVLLVILWLQLSWVWSQQKEVEQNSGPLSVPEGAIASLNCTYSDRGSQSFFWYRQYSGKSPELIMFIYSNGDKEDGRFTAQLNKASQYVSLLIRDSQPSDSATYLCAAVISNFGNEKLTFGTGTRLTIIPNIQNPDPAVYQLRDSKSSDKSVCLFTDFDSQTNVSQSKDSDVYITDKTVLDMRSMDFKSNSAVAWSNKSDFACANAFNNSIIPEDTFFPSPESSCDVKLVEKSFETDTNLNFQNLSVIGFRILLLKVAGFNLLMTLRLWSS

SEQ ID NO: 19 - protein, 5 aa, Homo sapiens
SGHRS

SEQ ID NO: 20 - protein, 6 aa, Homo sapiens
YFSETQ

SEQ ID NO: 21 - protein, 14 aa, Homo sapiens
CASSPWDSPNEQYF

SEQ ID NO: 22 - protein, 132 aa, Homo sapiens
MGSRLLCWVLLCLLGAGPVKAGVTQTPRYLIKTRGQQVTLSCSPISGHRSVSWYQQTPGQGLQFLFEYFSETQRNKGNFPGRFSGRQFSNSRSEMNVSTLELGDSALYLCASSPWDSPNEQYFGPGTRLTVT

SEQ ID NO: 23 - protein, 179 aa, Homo sapiens; identical to SEQ ID NO: 11

SEQ ID NO: 24 - protein, 311 aa, Homo sapiens
MGSRLLCWVLLCLLGAGPVKAGVTQTPRYLIKTRGQQVTLSCSPISGHRSVSWYQQTPGQGLQFLFEYFSETQRNKGNFPGRFSGRQFSNSRSEMNVSTLELGDSALYLCASSPWDSPNEQYFGPGTRLTVTEDLKNVFPPEVAVFEPSEAEISHTQKATLVCLATGFYPDHVELSWWVNGKEVHSGVSTDPQPLKEQPALNDSRYCLSSRLRVSATFWQNPRNHFRCQVQFYGLSENDEWTQDRAKPVTQIVSAEAWGRADCGFTSESYQQGVLSATILYEILLGKATLYAVLVSALVLMAMVKRKDSRG

SEQ ID NO: 25 - protein, 6 aa, Homo sapiens
NSAFQY

SEQ ID NO: 26 - skipped

SEQ ID NO: 27 - protein, 13 aa, Homo sapiens
CAMSEAAGNKLTF

SEQ ID NO: 28 - protein, 133 aa, Homo sapiens
MMKSLRVLLVILWLQLSWVWSQQKEVEQDPGPLSVPEGAIVSLNCTYSNSAFQYFMWYRQYSRKGPELLMYTYSSGNKEDGRFTAQVDKSSKYISLFIRDSQPSDSATYLCAMSEAAGNKLTFGGGTRVLVKP

SEQ ID NO: 29 - protein, 141 aa, Homo sapiens; identical to SEQ ID NO: 5

SEQ ID NO: 30 - protein, 274 aa, Homo sapiens
MMKSLRVLLVILWLQLSWVWSQQKEVEQDPGPLSVPEGAIVSLNCTYSNSAFQYFMWYRQYSRKGPELLMYTYSSGNKEDGRFTAQVDKSSKYISLFIRDSQPSDSATYLCAMSEAAGNKLTFGGGTRVLVKPNIQNPDPAVYQLRDSKSSDKSVCLFTDFDSQTNVSQSKDSDVYITDKTVLDMRSMDFKSNSAVAWSNKSDFACANAFNNSIIPEDTFFPSPESSCDVKLVEKSFETDTNLNFQNLSVIGFRILLLKVAGFNLLMTLRLWSS

SEQ ID NO: 31 - protein, 5 aa, Homo sapiens
SGHAT

SEQ ID NO: 32 - protein, 6 aa, Homo sapiens
FQNNGV

SEQ ID NO: 33 - protein, 13 aa, Homo sapiens
CASSYTNQGEAFF

SEQ ID NO: 34 - protein, 132 aa, Homo sapiens
MGTRLLCWAALCLLGAELTEAGVAQSPRYKIIEKRQSVAFWCNPISGHATLYWYQQILGQGPKLLIQFQNNGVVDDSQLPKDRFSAERLKGVDSTLKIQPAKLEDSAVYLCASSYTNQGEAFFGQGTRLTVV

SEQ ID NO: 35 - protein, 177 aa, Homo sapiens
EDLNKVFPPEVAVFEPSEAEISHTQKATLVCLATGFFPDHVELSWWVNGKEVHSGVSTDPQPLKEQPALNDSRYCLSSRLRVSATFWQNPRNHFRCQVQFYGLSENDEWTQDRAKPVTQIVSAEAWGRADCGFTSVSYQQGVLSATILYEILLGKATLYAVLVSALVLMAMVKRKDF

SEQ ID NO: 36 - protein, 309 aa, Homo sapiens
MGTRLLCWAALCLLGAELTEAGVAQSPRYKIIEKRQSVAFWCNPISGHATLYWYQQILGQGPKLLIQFQNNGVVDDSQLPKDRFSAERLKGVDSTLKIQPAKLEDSAVYLCASSYTNQGEAFFGQGTRLTVVEDLNKVFPPEVAVFEPSEAEISHTQKATLVCLATGFFPDHVELSWWVNGKEVHSGVSTDPQPLKEQPALNDSRYCLSSRLRVSATFWQNPRNHFRCQVQFYGLSENDEWTQDRAKPVTQIVSAEAWGRADCGFTSVSYQQGVLSATILYEILLGKATLYAVLVSALVLMAMVKRKDF

SEQ ID NO: 37 - protein, 6 aa, Homo sapiens
DRGSQS

SEQ ID NO: 38 - skipped

SEQ ID NO: 39 - protein, 13 aa, Homo sapiens
CAVLNQAGTALIF

SEQ ID NO: 40 - protein, 132 aa, Homo sapiens
MKSLRVLLVILWLQLSWVWSQQKEVEQNSGPLSVPEGAIASLNCTYSDRGSQSFFWYRQYSGKSPELIMSIYSNGDKEDGRFTAQLNKASQYVSLLIRDSQPSDSATYLCAVLNQAGTALIFGKGTTLSVSS

SEQ ID NO: 41 - protein, 141 aa, Homo sapiens; identical to SEQ ID NO: 5

SEQ ID NO: 42 - protein, 273 aa, Homo sapiens
MKSLRVLLVILWLQLSWVWSQQKEVEQNSGPLSVPEGAIASLNCTYSDRGSQSFFWYRQYSGKSPELIMSIYSNGDKEDGRFTAQLNKASQYVSLLIRDSQPSDSATYLCAVLNQAGTALIFGKGTTLSVSSNIQNPDPAVYQLRDSKSSDKSVCLFTDFDSQTNVSQSKDSDVYITDKTVLDMRSMDFKSNSAVAWSNKSDFACANAFNNSIIPEDTFFPSPESSCDVKLVEKSFETDTNLNFQNLSVIGFRILLLKVAGFNLLMTLRLWSS

SEQ ID NO: 43 - protein, 5 aa, Homo sapiens
SGDLS

SEQ ID NO: 44 - protein, 6 aa, Homo sapiens
YYNGEE

SEQ ID NO: 45 - protein, 17 aa, Homo sapiens
CASSAETGPWLGNEQFF

SEQ ID NO: 46 - protein, 135 aa, Homo sapiens
MGFRLLCCVAFCLLGAGPVDSGVTQTPKHLITATGQRVTLRCSPRSGDLSVYWYQQSLDQGLQFLIQYYNGEERAKGNILERFSAQQFPDLHSELNLSSLELGDSALYFCASSAETGPWLGNEQFFGPGTRLTVL

SEQ ID NO: 47 - protein, 179 aa, Homo sapiens; identical to SEQ ID NO: 11

SEQ ID NO: 48 - protein, 314 aa, Homo sapiens
MGFRLLCCVAFCLLGAGPVDSGVTQTPKHLITATGQRVTLRCSPRSGDLSVYWYQQSLDQGLQFLIQYYNGEERAKGNILERFSAQQFPDLHSELNLSSLELGDSALYFCASSAETGPWLGNEQFFGPGTRLTVLEDLKNVFPPEVAVFEPSEAEISHTQKATLVCLATGFYPDHVELSWWVNGKEVHSGVSTDPQPLKEQPALNDSRYCLSSRLRVSATFWQNPRNHFRCQVQFYGLSENDEWTQDRAKPVTQIVSAEAWGRADCGFTSESYQQGVLSATILYEILLGKATLYAVLVSALVLMAMVKRKDSRG

SEQ ID NO: 49 - protein, 7 aa, Homo sapiens
TSESDYY

SEQ ID NO: 50 - protein, 4 aa, Homo sapiens
QEAY

SEQ ID NO: 51 - protein, 15 aa, Homo sapiens
CAYRWAQGGSEKLVF

SEQ ID NO: 52 - protein, 136 aa, Homo sapiens
MACPGFLWALVISTCLEFSMAQTVTQSQPEMSVQEAETVTLSCTYDTSESDYYLFWYKQPPSRQMILVIRQEAYKQQNATENRFSVNFQKAAKSFSLKISDSQLGDAAMYFCAYRWAQGGSEKLVFGKGTKLTVNP

SEQ ID NO: 53 - protein, 141 aa, Homo sapiens
YIQKPDPAVYQLRDSKSSDKSVCLFTDFDSQTNVSQSKDSDVYITDKTVLDMRSMDFKSNSAVAWSNKSDFACANAFNNSIIPEDTFFPSPESSCDVKLVEKSFETDTNLNFQNLSVIGFRILLLKVAGFNLLMTLRLWSS

SEQ ID NO: 54 - protein, 277 aa, Homo sapiens
MACPGFLWALVISTCLEFSMAQTVTQSQPEMSVQEAETVTLSCTYDTSESDYYLFWYKQPPSRQMILVIRQEAYKQQNATENRFSVNFQKAAKSFSLKISDSQLGDAAMYFCAYRWAQGGSEKLVFGKGTKLTVNPYIQKPDPAVYQLRDSKSSDKSVCLFTDFDSQTNVSQSKDSDVYITDKTVLDMRSMDFKSNSAVAWSNKSDFACANAFNNSIIPEDTFFPSPESSCDVKLVEKSFETDTNLNFQNLSVIGFRILLLKVAGFNLLMTLRLWSS

SEQ ID NO: 55 - protein, 5 aa, Homo sapiens
MGHDK

SEQ ID NO: 56 - protein, 6 aa, Homo sapiens
SYGVNS

SEQ ID NO: 57 - protein, 16 aa, Homo sapiens
CATELWSSGGTGELFF

SEQ ID NO: 58 - protein, 134 aa, Homo sapiens
MTIRLLCYMGFYFLGAGLMEADIYQTPRYLVIGTGKKITLECSQTMGHDKMYWYQQDPGMELHLIHYSYGVNSTEKGDLSSESTVSRIRTEHFPLTLESARPSHTSQYLCATELWSSGGTGELFFGEGSRLTVL

SEQ ID NO: 59 - protein, 179 aa, Homo sapiens; identical to SEQ ID NO: 11

SEQ ID NO: 60 - protein, 313 aa, Homo sapiens
MTIRLLCYMGFYFLGAGLMEADIYQTPRYLVIGTGKKITLECSQTMGHDKMYWYQQDPGMELHLIHYSYGVNSTEKGDLSSESTVSRIRTEHFPLTLESARPSHTSQYLCATELWSSGGTGELFFGEGSRLTVLEDLKNVFPPEVAVFEPSEAEISHTQKATLVCLATGFYPDHVELSWWVNGKEVHSGVSTDPQPLKEQPALNDSRYCLSSRLRVSATFWQNPRNHFRCQVQFYGLSENDEWTQDRAKPVTQIVSAEAWGRADCGFTSESYQQGVLSATILYEILLGKATLYAVLVSALVLMAMVKRKDSRG

SEQ ID NO: 61 - protein, 6 aa, Homo sapiens
DRGSQS

SEQ ID NO: 62 - skipped

SEQ ID NO: 63 - protein, 13 aa, Homo sapiens
CAVGPSGTYKYIF

SEQ ID NO: 64 - protein, 132 aa, Homo sapiens
MKSLRVLLVILWLQLSWVWSQQKEVEQNSGPLSVPEGAIASLNCTYSDRGSQSFFWYRQYSGKSPELIMSIYSNGDKEDGRFTAQLNKASQYVSLLIRDSQPSDSATYLCAVGPSGTYKYIFGTGTRLKVLA

SEQ ID NO: 65 - protein, 141 aa, Homo sapiens; identical to SEQ ID NO: 5

SEQ ID NO: 66 - protein, 273 aa, Homo sapiens
MKSLRVLLVILWLQLSWVWSQQKEVEQNSGPLSVPEGAIASLNCTYSDRGSQSFFWYRQYSGKSPELIMSIYSNGDKEDGRFTAQLNKASQYVSLLIRDSQPSDSATYLCAVGPSGTYKYIFGTGTRLKVLANIQNPDPAVYQLRDSKSSDKSVCLFTDFDSQTNVSQSKDSDVYITDKTVLDMRSMDFKSNSAVAWSNKSDFACANAFNNSIIPEDTFFPSPESSCDVKLVEKSFETDTNLNFQNLSVIGFRILLLKVAGFNLLMTLRLWSS

SEQ ID NO: 67 - protein, 5 aa, Homo sapiens
MNHEY

SEQ ID NO: 68 - protein, 6 aa, Homo sapiens
SMNVEV

SEQ ID NO: 69 - protein, 14 aa, Homo sapiens
CASSPGGSGNEQFF

SEQ ID NO: 70 - protein, 132 aa, Homo sapiens
MGPQLLGYVVLCLLGAGPLEAQVTQNPRYLITVTGKKLTVTCSQNMNHEYMSWYRQDPGLGLRQIYYSMNVEVTDKGDVPEGYKVSRKEKRNFPLILESPSPNQTSLYFCASSPGGSGNEQFFGPGTRLTVL

SEQ ID NO: 71 - protein, 179 aa, Homo sapiens; identical to SEQ ID NO: 11

SEQ ID NO: 72 - protein, 311 aa, Homo sapiens
MGPQLLGYVVLCLLGAGPLEAQVTQNPRYLITVTGKKLTVTCSQNMNHEYMSWYRQDPGLGLRQIYYSMNVEVTDKGDVPEGYKVSRKEKRNFPLILESPSPNQTSLYFCASSPGGSGNEQFFGPGTRLTVLEDLKNVFPPEVAVFEPSEAEISHTQKATLVCLATGFYPDHVELSWWVNGKEVHSGVSTDPQPLKEQPALNDSRYCLSSRLRVSATFWQNPRNHFRCQVQFYGLSENDEWTQDRAKPVTQIVSAEAWGRADCGFTSESYQQGVLSATILYEILLGKATLYAVLVSALVLMAMVKRKDSRG

SEQ ID NO: 73 - protein, 6 aa, Homo sapiens
DRGSQS

SEQ ID NO: 74 - skipped

SEQ ID NO: 75 - protein, 14 aa, Homo sapiens
CAVVSGGGADGLTF

SEQ ID NO: 76 - protein, 133 aa, Homo sapiens
MKSLRVLLVILWLQLSWVWSQQKEVEQNSGPLSVPEGAIASLNCTYSDRGSQSFFWYRQYSGKSPELIMFIYSNGDKEDGRFTAQLNKASQYVSLLIRDSQPSDSATYLCAVVSGGGADGLTFGKGTHLIIQP

SEQ ID NO: 77 - protein, 141 aa, Homo sapiens; identical to SEQ ID NO: 53

SEQ ID NO: 78 - protein, 274 aa, Homo sapiens
MKSLRVLLVILWLQLSWVWSQQKEVEQNSGPLSVPEGAIASLNCTYSDRGSQSFFWYRQYSGKSPELIMFIYSNGDKEDGRFTAQLNKASQYVSLLIRDSQPSDSATYLCAVVSGGGADGLTFGKGTHLIIQPYIQKPDPAVYQLRDSKSSDKSVCLFTDFDSQTNVSQSKDSDVYITDKTVLDMRSMDFKSNSAVAWSNKSDFACANAFNNSIIPEDTFFPSPESSCDVKLVEKSFETDTNLNFQNLSVIGFRILLLKVAGFNLLMTLRLWSS

SEQ ID NO: 79 - protein, 5 aa, Homo sapiens
PRHDT

SEQ ID NO: 80 - protein, 6 aa, Homo sapiens
FYEKMQ

SEQ ID NO: 81 - protein, 14 aa, Homo sapiens
CASSLGRGGQPQHF

SEQ ID NO: 82 - protein, 142 aa, Homo sapiens
MLSPDLPDSAWNTRLLCHVMLCLLGAVSVAAGVIQSPRHLIKEKRETATLKCYPIPRHDTVYWYQQGPGQDPQFLISFYEKMQSDKGSIPDRFSAQQFSDYHSELNMSSLELGDSALYFCASSLGRGGQPQHFGDGTRLSIL

SEQ ID NO: 83 - protein, 177 aa, Homo sapiens; identical to SEQ ID NO: 35

SEQ ID NO: 84 - protein, 319 aa, Homo sapiens
MLSPDLPDSAWNTRLLCHVMLCLLGAVSVAAGVIQSPRHLIKEKRETATLKCYPIPRHDTVYWYQQGPGQDPQFLISFYEKMQSDKGSIPDRFSAQQFSDYHSELNMSSLELGDSALYFCASSLGRGGQPQHFGDGTRLSILEDLNKVFPPEVAVFEPSEAEISHTQKATLVCLATGFFPDHVELSWWVNGKEVHSGVSTDPQPLKEQPALNDSRYCLSSRLRVSATFWQNPRNHFRCQVQFYGLSENDEWTQDRAKPVTQIVSAEAWGRADCGFTSVSYQQGVLSATILYEILLGKATLYAVLVSALVLMAMVKRKDF

SEQ ID NO: 85 - protein, 6 aa, Homo sapiens
DSAIYN

SEQ ID NO: 86 - skipped

SEQ ID NO: 87 - protein, 15 aa, Homo sapiens
CAVRPTSGGSYIPTF

SEQ ID NO: 88 - protein, 133 aa, Homo sapiens
METLLGLLILWLQLQWVSSKQEVTQIPAALSVPEGENLVLNCSFTDSAIYNLQWFRQDPGKGLTSLLLIQSSQREQTSGRLNASLDKSSGRSTLYIAASQPGDSATYLCAVRPTSGGSYIPTFGRGTSLIVHP

SEQ ID NO: 89 - protein, 141 aa, Homo sapiens
YIQNPDPAVYQLRDSKSSDKSVCLFTDFDSQTNVSQSKDSDVYITDKTVLDMRSMDFKSNSAVAWSNKSDFACANAFNNSIIPEDTFFPSPESSCDVKLVEKSFETDTNLNFQNLSVIGFRILLLKVAGFNLLMTLRLWSS

SEQ ID NO: 90 - protein, 274 aa, Homo sapiens
METLLGLLILWLQLQWVSSKQEVTQIPAALSVPEGENLVLNCSFTDSAIYNLQWFRQDPGKGLTSLLLIQSSQREQTSGRLNASLDKSSGRSTLYIAASQPGDSATYLCAVRPTSGGSYIPTFGRGTSLIVHPYIQNPDPAVYQLRDSKSSDKSVCLFTDFDSQTNVSQSKDSDVYITDKTVLDMRSMDFKSNSAVAWSNKSDFACANAFNNSIIPEDTFFPSPESSCDVKLVEKSFETDTNLNFQNLSVIGFRILLLKVAGFNLLMTLRLWSS

SEQ ID NO: 91 - protein, 5 aa, Homo sapiens
MNHEY

SEQ ID NO: 92 - protein, 6 aa, Homo sapiens
SVGAGI

SEQ ID NO: 93 - protein, 14 aa, Homo sapiens
CASSYVGNTGELFF

SEQ ID NO: 94 - protein, 132 aa, Homo sapiens
MSIGLLCCAALSLLWAGPVNAGVTQTPKFQVLKTGQSMTLQCAQDMNHEYMSWYRQDPGMGLRLIHYSVGAGITDQGEVPNGYNVSRSTTEDFPLRLLSAAPSQTSVYFCASSYVGNTGELFFGEGSRLTVL

SEQ ID NO: 95 - protein, 179 aa, Homo sapiens; identical to SEQ ID NO: 11

SEQ ID NO: 96 - protein, 311 aa, Homo sapiens
MSIGLLCCAALSLLWAGPVNAGVTQTPKFQVLKTGQSMTLQCAQDMNHEYMSWYRQDPGMGLRLIHYSVGAGITDQGEVPNGYNVSRSTTEDFPLRLLSAAPSQTSVYFCASSYVGNTGELFFGEGSRLTVLEDLKNVFPPEVAVFEPSEAEISHTQKATLVCLATGFYPDHVELSWWVNGKEVHSGVSTDPQPLKEQPALNDSRYCLSSRLRVSATFWQNPRNHFRCQVQFYGLSENDEWTQDRAKPVTQIVSAEAWGRADCGFTSESYQQGVLSATILYEILLGKATLYAVLVSALVLMAMVKRKDSRG

SEQ ID NO: 97 - protein, 9 aa, Homo sapiens
SLLQHLIGL

SEQ ID NO: 98 - protein, 9 aa, Homo sapiens
ALLQHLIGL

SEQ ID NO: 99 - protein, 9 aa, Homo sapiens
SALQHLIGL

SEQ ID NO: 100 - protein, 9 aa, Homo sapiens
SLAQHLIGL

SEQ ID NO: 101 - protein, 9 aa, Homo sapiens
SLLAHLIGL

SEQ ID NO: 102 - protein, 9 aa, Homo sapiens
SLLQALIGL

SEQ ID NO: 103 - protein, 9 aa, Homo sapiens
SLLQHAIGL

SEQ ID NO: 104 - protein, 9 aa, Homo sapiens
SLLQHLAGL

SEQ ID NO: 105 - protein, 9 aa, Homo sapiens
SLLQHLIAL

SEQ ID NO: 106 - protein, 9 aa, Homo sapiens
SLLQHLIGA

SEQ ID NO: 107 - protein, 9 aa, Homo sapiens
TLLQHLIGL

SEQ ID NO: 108 - protein, 9 aa, Homo sapiens
STLQHLIGL

SEQ ID NO: 109 - protein, 9 aa, Homo sapiens
SLTQHLIGL

SEQ ID NO: 110 - protein, 9 aa, Homo sapiens
SLLTHLIGL

SEQ ID NO: 111 - protein, 9 aa, Homo sapiens
SLLQTLIGL

SEQ ID NO: 112 - protein, 9 aa, Homo sapiens
SLLQHTIGL

SEQ ID NO: 113 - protein, 9 aa, Homo sapiens
SLLQHLTGL

SEQ ID NO: 114 - protein, 9 aa, Homo sapiens
SLLQHLITL

SEQ ID NO: 115 - protein, 9 aa, Homo sapiens
SLLQHLIGT

SEQ ID NO: 116 - protein, 9 aa, Homo sapiens
SILQTLILV

SEQ ID NO: 117 - protein, 9 aa, Homo sapiens
SLIEHLQGL

SEQ ID NO: 118 - protein, 9 aa, Homo sapiens
SLIQHLEEI

SEQ ID NO: 119 - protein, 9 aa, Homo sapiens
SLLKNLIYL

SEQ ID NO: 120 - protein, 9 aa, Homo sapiens
SLLNHLPYL

SEQ ID NO: 121 - protein, 9 aa, Homo sapiens
SLLQHVLLL

SEQ ID NO: 122 - protein, 9 aa, Homo sapiens
SLLQKQIML

SEQ ID NO: 123 - protein, 9 aa, Homo sapiens
SLSQELVGV

SEQ ID NO: 124 - protein, 9 aa, Homo sapiens
SVLGALIGV

SEQ ID NO: 125 - protein, 9 aa, Homo sapiens
VLLHHQIGL

SEQ ID NO: 126 - protein, 9 aa, Homo sapiens
SLLMWITQV

SEQ ID NO: 127 - protein, 6 aa, Homo sapiens
SSNFYA

SEQ ID NO: 128 - skipped

SEQ ID NO: 129 - protein, 11 aa, Homo sapiens
CALYNNNDMRF

SEQ ID NO: 130 - protein, 132 aa, Homo sapiens
MEKNPLAAPLLILWFHLDCVSSILNVEQSPQSLHVQEGDSTNFTCSFPSSNFYALHWYRKETAKSPEALFVMTLNGDEKKKGRISATLNTKEGYSYLYIKGSQPEDSATYLCALYNNNDMRFGAGTRLTVKP

SEQ ID NO: 131 - protein, 141 aa, Homo sapiens; identical to SEQ ID NO: 5

SEQ ID NO: 132 - protein, 273 aa, Homo sapiens
MEKNPLAAPLLILWFHLDCVSSILNVEQSPQSLHVQEGDSTNFTCSFPSSNFYALHWYRKETAKSPEALFVMTLNGDEKKKGRISATLNTKEGYSYLYIKGSQPEDSATYLCALYNNNDMRFGAGTRLTVKPNIQNPDPAVYQLRDSKSSDKSVCLFTDFDSQTNVSQSKDSDVYITDKTVLDMRSMDFKSNSAVAWSNKSDFACANAFNNSIIPEDTFFPSPESSCDVKLVEKSFETDTNLNFQNLSVIGFRILLLKVAGFNLLMTLRLWSS

SEQ ID NO: 133 - protein, 5 aa, Homo sapiens
SGHNS

SEQ ID NO: 134 - protein, 6 aa, Homo sapiens
FNNNVP

SEQ ID NO: 135 - protein, 13 aa, Homo sapiens
CASSPGSTDTQYF

SEQ ID NO: 136 - protein, 132 aa, Homo sapiens
MDSWTFCCVSLCILVAKHTDAGVIQSPRHEVTEMGQEVTLRCKPISGHNSLFWYRETMMRGLELLIYFNNNVPIDDSGMPEDRFSAKMPNASFSTLKIQPSEPRDSAVYFCASSPGSTDTQYFGPGTRLTVL

SEQ ID NO: 137 - protein, 179 aa, Homo sapiens; identical to SEQ ID NO: 11

SEQ ID NO: 138 - protein, 311 aa, Homo sapiens
MDSWTFCCVSLCILVAKHTDAGVIQSPRHEVTEMGQEVTLRCKPISGHNSLFWYRETMMRGLELLIYFNNNVPIDDSGMPEDRFSAKMPNASFSTLKIQPSEPRDSAVYFCASSPGSTDTQYFGPGTRLTVLEDLKNVFPPEVAVFEPSEAEISHTQKATLVCLATGFYPDHVELSWWVNGKEVHSGVSTDPQPLKEQPALNDSRYCLSSRLRVSATFWQNPRNHFRCQVQFYGLSENDEWTQDRAKPVTQIVSAEAWGRADCGFTSESYQQGVLSATILYEILLGKATLYAVLVSALVLMAMVKRKDSRG

SEQ ID NO: 139 - protein, 9 aa, Homo sapiens
LLLVHLIPV

SEQ ID NO: 140 - protein, 9 aa, Homo sapiens
IILRHLIEI

SEQ ID NO: 141 - protein, 9 aa, Homo sapiens
KILLHLIHI

SEQ ID NO: 142 - protein, 9 aa, Homo sapiens
KVLPHLIPL

SEQ ID NO: 143 - protein, 9 aa, Homo sapiens
SALVHLIPV

SEQ ID NO: 144 - protein, 9 aa, Homo sapiens
NALVHLIEV

SEQ ID NO: 145 - protein, 9 aa, Homo sapiens
VALGHLIGI

SEQ ID NO: 146 - protein, 9 aa, Homo sapiens
NALVHLIEI

SEQ ID NO: 147 - protein, 9 aa, Homo sapiens
WALGHLIGI

SEQ ID NO: 148 - protein, 9 aa, Homo sapiens
QALEHLIYI

SEQ ID NO: 149 - protein, 9 aa, Homo sapiens
ISLAHLILV

SEQ ID NO: 150 - protein, 9 aa, Homo sapiens
ETLDHLISL

SEQ ID NO: 151 - protein, 9 aa, Homo sapiens
ALLSHLICR

SEQ ID NO: 152 - protein, 9 aa, Homo sapiens
KELRHLIEV

SEQ ID NO: 153 - protein, 9 aa, Homo sapiens
IALVHLIMV

SEQ ID NO: 154 - protein, 9 aa, Homo sapiens
CWLCHLIKL

SEQ ID NO: 155 - protein, 9 aa, Homo sapiens
GKLTHLIPV

SEQ ID NO: 156 - protein, 9 aa, Homo sapiens
HLLMHLIGS

SEQ ID NO: 157 - protein, 9 aa, Homo sapiens
TQLDHLIPG

SEQ ID NO: 158 - protein, 9 aa, Homo sapiens
QDLWHLIKL

SEQ ID NO: 159 - protein, 9 aa, Homo sapiens
IALKHLIPT

SEQ ID NO: 160 - protein, 9 aa, Homo sapiens
IALKHLILT

SEQ ID NO: 161 - protein, 9 aa, Homo sapiens
LQLIHLINV

SEQ ID NO: 162 - protein, 9 aa, Homo sapiens
SQLVHLIYV

SEQ ID NO: 163 - protein, 9 aa, Homo sapiens
CLLPHLIQH

SEQ ID NO: 164 - protein, 9 aa, Homo sapiens
MVLVHLIHS

SEQ ID NO: 165 - protein, 9 aa, Homo sapiens
SDLFHLIGV

SEQ ID NO: 166 - protein, 9 aa, Homo sapiens
KLLFHLIQS

SEQ ID NO: 167 - protein, 9 aa, Homo sapiens
KLLLHLIQS

SEQ ID NO: 168 - protein, 9 aa, Homo sapiens
SFLVHLIGL

SEQ ID NO: 169 - protein, 9 aa, Homo sapiens
YGLKHLISV

SEQ ID NO: 170 - protein, 9 aa, Homo sapiens
SELPHLIGI

SEQ ID NO: 171 - protein, 9 aa, Homo sapiens
YALSHLIHA

SEQ ID NO: 172 - protein, 9 aa, Homo sapiens
TLLGHLISK

SEQ ID NO: 173 - protein, 9 aa, Homo sapiens
SQLSHLIAM

SEQ ID NO: 174 - protein, 9 aa, Homo sapiens
FFLVHLICM

SEQ ID NO: 175 - protein, 9 aa, Homo sapiens
VSLHHLINA

SEQ ID NO: 176 - protein, 9 aa, Homo sapiens
IMLIHLIRL

SEQ ID NO: 177 - protein, 9 aa, Homo sapiens
ITLIHLIRL

SEQ ID NO: 178 - protein, 9 aa, Homo sapiens
SELFHLIPL

SEQ ID NO: 179 - protein, 9 aa, Homo sapiens
SVLFHLIPL

SEQ ID NO: 180 - protein, 9 aa, Homo sapiens
AQLAHLILS

SEQ ID NO: 181 - protein, 9 aa, Homo sapiens
FLLGHLIPR

SEQ ID NO: 182 - protein, 9 aa, Homo sapiens
MLLGHLIFF

SEQ ID NO: 183 - protein, 9 aa, Homo sapiens
VLLFHLIEE

SEQ ID NO: 184 - protein, 9 aa, Homo sapiens
VFLRHLITL

SEQ ID NO: 185 - protein, 9 aa, Homo sapiens
TLLDHLIFK

SEQ ID NO: 186 - protein, 9 aa, Homo sapiens
SVLVHLIPA

SEQ ID NO: 187 - protein, 9 aa, Homo sapiens
AKLEHLIYL

SEQ ID NO: 188 - protein, 9 aa, Homo sapiens
SLLPHLILS

SEQ ID NO: 189 - protein, 9 aa, Homo sapiens
SILGHLICS

SEQ ID NO: 190 - protein, 9 aa, Homo sapiens
QSLEHLIYI

SEQ ID NO: 191 - protein, 9 aa, Homo sapiens
YILNHLINP

SEQ ID NO: 192 - protein, 9 aa, Homo sapiens
YKLLHLIWI

SEQ ID NO: 193 - protein, 9 aa, Homo sapiens
KLLCHLIEH

SEQ ID NO: 194 - protein, 9 aa, Homo sapiens
ALLDHLITH

SEQ ID NO: 195 - protein, 9 aa, Homo sapiens
FMLSHLIQH

SEQ ID NO: 196 - protein, 7 aa, Homo sapiens
MTLNGDE

SEQ ID NO: 197 - protein, 6 aa, Homo sapiens
IYSNGD

SEQ ID NO: 198 - protein, 6 aa, Homo sapiens
TYSSGN

SEQ ID NO: 199 - protein, 6 aa, Homo sapiens
IYSNGD

SEQ ID NO: 200 - protein, 7 aa, Homo sapiens
QEAYKQQ

SEQ ID NO: 201 - protein, 6 aa, Homo sapiens
IYSNGD

SEQ ID NO: 202 - protein, 6 aa, Homo sapiens
IYSNGD

SEQ ID NO: 203 - protein, 7 aa, Homo sapiens
IQSSQRE

SEQ ID NO: 204 - protein, 7 aa, Homo sapiens
MTLNGDE